European Patent Specification EP 3 894 590 B1, published October 22, 2025. Title: METHODS OF USING MASTER/COPY ARRAYS FOR SPATIAL DETECTION. Applicant: 10x Genomics, Inc. The sequence listing filed with the application follows.

SEQUENCE LISTING (7 sequences)

SEQ ID NO: 1 - protein, 16 aa, Artificial
  Synthetic Trademark of PURAMATRIX polypeptide sequence
RADARADARADARADA

SEQ ID NO: 2 - protein, 16 aa, Artificial
  Synthetic EAK16 polypeptide sequence
AEAEAKAKAEAEAKAK

SEQ ID NO: 3 - protein, 12 aa, Artificial
  Synthetic KLD12 polypeptide sequence
KLDLKLDLKLDL

SEQ ID NO: 4 - DNA, 18 bp, Artificial
  18s cDNA Probe 1
gaggaattcccagtaagt

SEQ ID NO: 5 - DNA, 18 bp, Artificial
  18S cDNA Probe 2
gagattgagcaataacag

SEQ ID NO: 6 - DNA, 18 bp, Artificial
  18s cDNA Probe 3
gtagttccgaccataaac

SEQ ID NO: 7 - DNA, 18 bp, Artificial
  18s cDNA Probe 4
ggtgactctagataacct